European Patent Specification EP 3 271 390 B1, published September 27, 2023. Title: A Serotype Cross-Reactive Dengue Antibody And Uses Thereof. Applicant: AGENCY FOR SCIENCE, TECHNOLOGY AND RESEARCH NATIONAL UNIVERSITY OF SINGAPORE. The sequence listing filed with the application follows.

SEQUENCE LISTING (12 sequences)

SEQ ID NO: 1 - DNA, 396 bp, Artificial Sequence
  Synthetic sequence
  misc_feature: Heavy chain variable region
gaggtccagctggtacagtctgggcctgacgtcgagaagcctggggcctcagtgaaggtttcctgcaaggcatctggatacaccttcaccagcaactatatacactgggtgcgacaggcccctggacaagggcttgagtggatgggggtaatcaaccctaggggtggtagcacagccagcgcacagaaattccagggaagaatcaccatgaccagggacacgtccacgagcacagtttacatggaactgagcagcctgagatctgacgacacggccgtgtattactgtgcgagagggggaagggcccttttctatgatagttacacgaccccccgagacggagggtcgtggtggttcgacccctggggccagggaagcctggtcaccgtctcctca

SEQ ID NO: 2 - DNA, 324 bp, Artificial sequence
  Synthetic sequence
  misc_feature: Light chain variable region
gacatccagttgacccagtctccatcttccctgtctgcatctgtaggagacagagtcaccttcacttgccaggcgagccaggacattaggaagtatttaaattggtatcagcagaaaccagggaaagcccctaaactcctaatctacgatgcatccaatttgaaaacaggggtcccatcaaggttcagtggaagtggatctgggacagattttactttcaccatcagcagcctgcagcctgaagatgttgcaacatactactgtcaacagtttgatgatctcccgatcaccttcggccaggggacacgactgcagattaaacga

SEQ ID NO: 3 - protein, 8 aa, Artificial sequence
  Synthetic sequence
  MISC_FEATURE: CDRH1
GYTFTSNY

SEQ ID NO: 4 - protein, 8 aa, Artificial sequence
  Synthetic sequence
  MISC_FEATURE: CDRH2
INPRGGST

SEQ ID NO: 5 - protein, 25 aa, Artificial sequence
  Synthetic sequence
  MISC_FEATURE: CDRH3
ARGGRALFYDSYTTPRDGGSWWFDP

SEQ ID NO: 6 - protein, 6 aa, Artificial sequence
  Synthetic sequence
  MISC_FEATURE: CDRL1
QDIRKY

SEQ ID NO: 7 - protein, 4 aa, Artificial sequence
  Synthetic sequence
  MISC_FEATURE: CDRL2
  misc_feature (4)..(4): Xaa can be any naturally occurring amino acid
DASX

SEQ ID NO: 8 - protein, 9 aa, Artificial sequence
  Synthetic sequence
  MISC_FEATURE: CDRL3
QQFDDLPIT

SEQ ID NO: 9 - protein, 132 aa, Artificial sequence
  Synthetic sequence
  MISC_FEATURE: Heavy chain variable region
EVQLVQSGPDVEKPGASVKVSCKASGYTFTSNYIHWVRQAPGQGLEWMGVINPRGGSTASAQKFQGRITMTRDTSTSTVYMELSSLRSDDTAVYYCARGGRALFYDSYTTPRDGGSWWFDPWGQGSLVTVSS

SEQ ID NO: 10 - protein, 107 aa, Artificial sequence
  Synthetic sequence
  MISC_FEATURE: Light chain variable region
DIQLTQSPSSLSASVGDRVTFTCQASQDIRKYLNWYQQKPGKAPKLLIYDASNLKTGVPSRFSGSGSGTDFTFTISSLQPEDVATYYCQQFDDLPITFGQGTRLQIK

SEQ ID NO: 11 - DNA, 984 bp, Artificial sequence
  Synthetic sequence
  misc_feature: 3C H5L1 heavy chain constant region with LALA mutation
gcttccaccaagggcccatcggtcttccccctggcaccctcctccaagtcgacctctgggggcacagcggccctgggctgcctggtcaaggactacttccccgaaccggtgacggtgtcgtggaactcaggcgccctgaccagtggcgtgcacaccttcccggctgtcctacagtcctcaggactctactccctcagtagtgtggtgaccgtgccctccagtagtttgggcacccagacctacatctgcaacgtgaatcacaagcccagtaacaccaaggtggacaagagagttgagcccaaatcttgtgacaaaactcacacatgcccaccgtgcccagcacctgaggccgccgggggaccgtcagtcttcctcttccccccaaaacccaaggacaccctcatgatctcccggacccctgaggtcacatgcgtggtggtggacgtgagtcacgaagaccctgaggtcaagttcaactggtacgtggacggcgtggaggtgcataatgccaagacaaagccgcgggaggagcagtacaacagtacgtaccgtgtggtcagtgtcctcaccgtcctgcaccaggactggctgaatggcaaggagtacaagtgcaaggtctccaacaaagccctcccagcccccatcgagaaaaccatctccaaagccaaagggcagccccgagaaccacaggtgtacaccctgcccccatcccgggaggagatgaccaagaaccaggtcagtctgacctgcctggtcaaaggcttctatcccagtgacatcgccgtggagtgggagagtaatgggcagccggagaacaactacaagaccacgcctcccgtgctggactccgacggctccttcttcctctacagtaagctcaccgtggacaagagtaggtggcagcaggggaacgtcttctcatgctccgtgatgcatgaggctctgcacaaccactacacgcagaagagtctctccctgtctccg

SEQ ID NO: 12 - protein, 328 aa, Artificial sequence
  Synthetic sequence
  MISC_FEATURE: 3C H5L1 heavy chain constant region with LALA mutation
  MISC_FEATURE (117)..(118): LALA mutation
ASTKGPSVFPLAPSSKSTSGGTAALGCLVKDYFPEPVTVSWNSGALTSGVHTFPAVLQSSGLYSLSSVVTVPSSSLGTQTYICNVNHKPSNTKVDKRVEPKSCDKTHTCPPCPAPEAAGGPSVFLFPPKPKDTLMISRTPEVTCVVVDVSHEDPEVKFNWYVDGVEVHNAKTKPREEQYNSTYRVVSVLTVLHQDWLNGKEYKCKVSNKALPAPIEKTISKAKGQPREPQVYTLPPSREEMTKNQVSLTCLVKGFYPSDIAVEWESNGQPENNYKTTPPVLDSDGSFFLYSKLTVDKSRWQQGNVFSCSVMHEALHNHYTQKSLSLSP